European Patent Application EP 4 174 086 A1, published May 3, 2023. Title: Antibody specifically binding to LGALS3BP and use thereof. Applicant: University of Ulsan Foundation For Industry Cooperation THE ASAN FOUNDATION. The sequence listing filed with the application follows.

SEQUENCE LISTING (24 sequences)

SEQ ID NO: 1 - protein, 10 aa, Artificial Sequence
  #67 heavy chain CDR1
GFTFSSYGLG

SEQ ID NO: 2 - protein, 16 aa, Artificial Sequence
  #67 heavy chain CDR2
GISSGGATFYGAAMKG

SEQ ID NO: 3 - protein, 16 aa, Artificial Sequence
  #67 heavy chain CDR3
DARSGSWSPDAGQIDA

SEQ ID NO: 4 - protein, 9 aa, Artificial Sequence
  #67 light chain CDR1
SGSSGSHYG

SEQ ID NO: 5 - protein, 7 aa, Artificial Sequence
  #67 light chain CDR2
SNDKRPS

SEQ ID NO: 6 - protein, 8 aa, Artificial Sequence
  #67 light chain CDR3
GSIDSSGI

SEQ ID NO: 7 - protein, 126 aa, Artificial Sequence
  #67 VH
AVTLDESGGGLQTPGGALSLVCKGSGFTFSSYGLGWVRQAPGKGLEYVAGISSGGATFYGAAMKGRATISRDNGQSTVRLQLNNLRAEDTATYYCAKDARSGSWSPDAGQIDAWGHGTEVIVSSTS

SEQ ID NO: 8 - protein, 101 aa, Artificial Sequence
  #67 VL
LTQPSSVSANLGGTVEITCSGSSGSHYGWFQQKSPGSAPVTLIYSNDKRPSDIPSRFSGSKSGSTATLTITGVQAEDEAVYFCGSIDSSGIFGAGTTLTVL

SEQ ID NO: 9 - protein, 10 aa, Artificial Sequence
  #84 heavy chain CDR1
GFTFNGYGMN

SEQ ID NO: 10 - protein, 17 aa, Artificial Sequence
  #84 heavy chain CDR2
GIDDTGSYTAYAPAVRG

SEQ ID NO: 11 - protein, 13 aa, Artificial Sequence
  #84 heavy chain CDR3
GYGDVWGGDEIDA

SEQ ID NO: 12 - protein, 8 aa, Artificial Sequence
  #84 light chain CDR1
SGGSSGYG

SEQ ID NO: 13 - protein, 7 aa, Artificial Sequence
  #84 light chain CDR2
DNDKRPS

SEQ ID NO: 14 - protein, 9 aa, Artificial Sequence
  #84 light chain CDR3
GGYDNSVGI

SEQ ID NO: 15 - protein, 124 aa, Artificial Sequence
  #84 VH
AVTLDESGGGLQTPGGALSLVCKASGFTFNGYGMNWVRQAPGKGLEWVAGIDDTGSYTAYAPAVRGRATISRDNGQSTVRLQLNNLRAEDTATYYCAKGYGDVWGGDEIDAWGHGTEVIVSSTS

SEQ ID NO: 16 - protein, 101 aa, Artificial Sequence
  #84 VL
LTQPSSVSANLGGTVKITCSGGSSGYGWHQQKSPGSAPVTVIYDNDKRPSDIPSRFSGSLSGSTNTLTITGVQAEDEAVYFCGGYDNSVGIFGAGTTLTVL

SEQ ID NO: 17 - DNA, 378 bp, Artificial Sequence
  #67 VH
gccgtgacgttggacgagtccgggggcggcctccagacgcccggaggagcgctcagcctcgtctgcaagggctccgggttcaccttcagcagttatggcctgggttgggtgcgacaggcgcccggcaaggggctcgagtacgttgcgggtattagtagcggtggtgcaacattctacggggcggcgatgaagggccgtgccaccatctcgagggacaacgggcagagcacagtgaggctgcagctgaacaacctcagggctgaggacaccgccacctactactgcgccaaagatgctcgcagtggtagttggagtcctgatgctggtcaaatcgacgcatggggccacgggaccgaagtcatcgtctcctccactagt

SEQ ID NO: 18 - DNA, 303 bp, Artificial Sequence
  #67 VL
ctgactcagccgtcctcggtgtcagcaaacctgggaggaaccgtcgagatcacctgctccgggagtagtggcagccactatggctggttccagcagaagtcacctggcagtgcccctgtcactctgatctatagcaacgacaagagaccctcggacatcccttcacgattctccggttccaaatccggctccacagccacattaaccatcactggggtccaagccgaggacgaggctgtctatttctgtgggagcatagacagcagtggtatatttggggccgggacaaccctgaccgtccta

SEQ ID NO: 19 - DNA, 369 bp, Artificial Sequence
  #84 VH
gtgacgttggacgagtccgggggcggcctccagacgcccggaggagcgctcagcctcgtctgcaaggcctccgggttcaccttcaacggttacggcatgaactgggtgcgacaggcgcccggcaaggggctggagtgggtcgctggtattgatgacactggtagttacacagcatacgcgccggcggtgaggggccgtgccaccatctcgagggacaacgggcagagcacagtgaggctgcagctgaacaacctcagggctgaggacaccgccacctactactgcgccaaaggttatggtgatgtttggggtggtgatgagatcgacgcatggggccacgggaccgaagtcatcgtctcctccactagt

SEQ ID NO: 20 - DNA, 303 bp, Artificial Sequence
  #84 VL
ctgactcagccgtcctcggtgtcagcaaacctgggaggaaccgtcaagatcacctgctccgggggtagcagcggctatggctggcaccagcagaaatcacctggcagtgcccctgtcactgtgatctatgacaacgacaagagaccctcggacatcccttcacgattctccggttccctatccggctccacaaacacattaaccatcactggggtccaagccgaggacgaggctgtctatttctgtggtggctacgacaacagtgtcggtatatttggggccgggacaaccctgaccgtccta

SEQ ID NO: 21 - protein, 122 aa, Artificial Sequence
  Humanized #84 VH7
QVQLVESGGGVVQPGGSLRLSCAASGFTFNGYGMNWVRQAPGKGLEWVSGIDDTGSYTAYAPAVRGRFTISRDNSKNTLYLQMNSLRAEDTAVYYCAKGYGDVWGGDEIDAWGQGTLVTVSS

SEQ ID NO: 22 - protein, 101 aa, Artificial Sequence
  Humanized #84 VL11
ELTQPPSVSVSPGQTARITCSGGSSGYGWHQQKPGQAPVLVIYDNDKRPSGIPERFSGSSSGTTVTLTISGVQAEDEADYYCGGYDNSVGIFGGGTKLTVL

SEQ ID NO: 23 - protein, 101 aa, Artificial Sequence
  Humanized #84 VL12
ELTQPPSVSVSPGQTARITCSGGSSGYGWHQQKPGQAPVLVIYDNDKRPSGIPERFSGSLSGTTVTLTISGVQAEDEADYYCGGYDNSVGIFGGGTKLTVL

SEQ ID NO: 24 - protein, 101 aa, Artificial Sequence
  Humanized #84 VL13
ELTQPPSVSVSPGQTARITCSGGSSGYGWHQQKPGQAPVLVIYDNDKRPSGIPERFSGSSSGSTVTLTISGVQAEDEADYYCGGYDNSVGIFGGGTKLTVL